European Patent Application EP 4 159 859 A1, published April 5, 2023. Title: anti-human NR1 antibody derivatives. Applicant: Astellas Pharma Inc. The sequence listing filed with the application follows.

SEQUENCE LISTING (50 sequences)

SEQ ID NO: 1 - DNA, 360 bp, Artificial Sequence
  codon optimized
  CDS (1)..(360)
caggtccagctgcaagagtctggccctggactggtcaagccttctggcaccctgtctctgacatgtgctgtgtccggcggctccatctcctcctctaattggtggtcttgggtccgacagcctcctggcaaaggactggaatggatcggcgagatctaccactccggcaacaccaactacaaccccagcctgaagtccagagtgaccgtgtccgtggacaagtccaagaaccagttctccctgaagctgacctctgtgaccgctgccgataccgccgtgtactactgtgctagagatgtgtctggcggagtgaattggttcgatccttggggccagggcacactggttaccgtgtcctct

SEQ ID NO: 2 - protein, 120 aa, Homo sapiens
QVQLQESGPGLVKPSGTLSLTCAVSGGSISSSNWWSWVRQPPGKGLEWIGEIYHSGNTNYNPSLKSRVTVSVDKSKNQFSLKLTSVTAADTAVYYCARDVSGGVNWFDPWGQGTLVTVSS

SEQ ID NO: 3 - DNA, 330 bp, Artificial Sequence
  codon optimized
  CDS (1)..(330)
aactttatgctgacccagcctcactccgtgtccgagtctccaggcaagaccgtgaccatctcctgtaccagatcctccggctctatcgcctccaactacgtgcagtggtatcagcagaggcctggctctgctcctaccaccgtgatctacgaggacaaccagaggccttctggcgtgcccgataggttctctggctccatcgactcctcttccaactccgcctctctgaccatcagcggcctgaaaaccgaggacgaggccgactactactgccagtcctacgactcttccaccgtggtgtttggcggcggaacaaagctgacagtgctg

SEQ ID NO: 4 - protein, 110 aa, Homo sapiens
NFMLTQPHSVSESPGKTVTISCTRSSGSIASNYVQWYQQRPGSAPTTVIYEDNQRPSGVPDRFSGSIDSSSNSASLTISGLKTEDEADYYCQSYDSSTVVFGGGTKLTVL

SEQ ID NO: 5 - DNA, 363 bp, Artificial Sequence
  mouse antibody/ humanized
  CDS (1)..(363)
gaagttcagctggttcagtctggcgccgaagtgaagaagcctggcgagtccctgaagatctcctgcaaaggctccggctacacctacaccagctactggatgaactgggtccgacagatgcctggcaaaggcctggaatggatgggcagaatcgacccctacgactccgagacacactacgaccagaaattcaaggaccaagtgaccctgagcgtggacaagtccatctccaccgcttacctgcagtggtcctctctgaaggcctctgacaccgccatgtactactgtgctggcggcatcaccaccatcctcggcggctactttgattactggggccagggcacactggtcaccgtttcttcc

SEQ ID NO: 6 - protein, 121 aa, Artificial Sequence
  Synthetic Construct
EVQLVQSGAEVKKPGESLKISCKGSGYTYTSYWMNWVRQMPGKGLEWMGRIDPYDSETHYDQKFKDQVTLSVDKSISTAYLQWSSLKASDTAMYYCAGGITTILGGYFDYWGQGTLVTVSS

SEQ ID NO: 7 - DNA, 327 bp, Artificial Sequence
  mouse antibody/ humanized
  CDS (1)..(327)
gacatccagatgacccagtctccatcctctctgtccgcctctgtgggcgacagagtgaccatcacctgtagagccagccaggacatctccaactacctgaactggtatcagcagaagcccggcaaggcccctaagctgctgatctactacacctctcggctgcactctggcgtgccctctagattttctggctccggctctggcaccgactataccctgacaatctccagcctgcagcctgaggacttcgccacctactattgccagcagggcaacaccctgcctccatacacatttggccagggcaccaaggtggaaatcaagcgt

SEQ ID NO: 8 - protein, 109 aa, Artificial Sequence
  Synthetic Construct
DIQMTQSPSSLSASVGDRVTITCRASQDISNYLNWYQQKPGKAPKLLIYYTSRLHSGVPSRFSGSGSGTDYTLTISSLQPEDFATYYCQQGNTLPPYTFGQGTKVEIKR

SEQ ID NO: 9 - DNA, 366 bp, Artificial Sequence
  mouse antibody/ humanized
  CDS (1)..(366)
gaagtgcagctggttgaatctggcggcggattggttcagcctggcggatctctgagactgtcctgcaaggcttctggctacgcctacacctcctactggatgaactgggtccgacaggctcctggcaaaggactcgtgtgggtcggaagaatcgacccctacgactccgagacacactacaaccagaagttcaaggaccggttcaccctgagcgtggacaaggccaagtctaccacctacctgcagatgaactccctgagagccgaggacaccgccgtgtactattgcgctaccctgatcaccacactgagaggcgagggcgccatggaatattggggacagggaaccctggtcaccgtgtcctct

SEQ ID NO: 10 - protein, 122 aa, Artificial Sequence
  Synthetic Construct
EVQLVESGGGLVQPGGSLRLSCKASGYAYTSYWMNWVRQAPGKGLVWVGRIDPYDSETHYNQKFKDRFTLSVDKAKSTTYLQMNSLRAEDTAVYYCATLITTLRGEGAMEYWGQGTLVTVSS

SEQ ID NO: 11 - DNA, 324 bp, Artificial Sequence
  mouse antibody/ humanized
  CDS (1)..(324)
gacctgcagatgacccagtctccttccagcctgtctgcctctgtgggcgacagagtgaccatcacatgcaaggccagccaggacgtgaacaccgccgttgcttggtatcagcagaagcctggcaaggcccctaagctgctgatctactgggcctccaccagacataccggcgtgccctctagattctccggctctggctctggcaccgactataccctgacaatctccagcctgcagcctgaggacttcgccacctactactgccagcagcactacagcacccctttcacctttggccagggcaccaaggtggaaatcaagcgt

SEQ ID NO: 12 - protein, 108 aa, Artificial Sequence
  Synthetic Construct
DLQMTQSPSSLSASVGDRVTITCKASQDVNTAVAWYQQKPGKAPKLLIYWASTRHTGVPSRFSGSGSGTDYTLTISSLQPEDFATYYCQQHYSTPFTFGQGTKVEIKR

SEQ ID NO: 13 - DNA, 357 bp, Artificial Sequence
  mouse antibody/ humanized
  CDS (1)..(357)
caggttcagctgcaagagtctggccctggcctggtcaagccttccgaaacactgtccctgacctgcagcgtgaccggctactctatcacctccgactactactggcactggatcagacagcctccaggcaaaggcctggaatggatcgcctacatcagatacgacggccggaacgactacaaccccagcctgaagaacagagtgaccatcagccgggacacctccaagaaccagttctccctgaagctgtcctccgtgaccgctgctgataccgccgtgtactactgcgccagagaggactacggctcctcctcctttgattactggggccagggcaccctggtcaccgttagttct

SEQ ID NO: 14 - protein, 119 aa, Artificial Sequence
  Synthetic Construct
QVQLQESGPGLVKPSETLSLTCSVTGYSITSDYYWHWIRQPPGKGLEWIAYIRYDGRNDYNPSLKNRVTISRDTSKNQFSLKLSSVTAADTAVYYCAREDYGSSSFDYWGQGTLVTVSS

SEQ ID NO: 15 - DNA, 324 bp, Artificial Sequence
  mouse antibody/ humanized
  CDS (1)..(324)
gacatccagatgacccagtctccatcctctctgtccgcctctgtgggcgacagagtgaccatcacctgtcgggcctccgagaacatctactccaacctggcctggtatcagcagaagcctggcaaggctcctaagctgctggtgtacgccgctaccaatctggctgatggcgtgccctctagattctccggctctggctctggcaccgactataccctgacaatctccagcctgcagcctgaggacttcgccacctactactgccagcacttctgggacagccctccaacctttggccagggcaccaaggtggaaatcaagcgt

SEQ ID NO: 16 - protein, 108 aa, Artificial Sequence
  Synthetic Construct
DIQMTQSPSSLSASVGDRVTITCRASENIYSNLAWYQQKPGKAPKLLVYAATNLADGVPSRFSGSGSGTDYTLTISSLQPEDFATYYCQHFWDSPPTFGQGTKVEIKR

SEQ ID NO: 17 - DNA, 357 bp, Artificial Sequence
  mouse antibody/ humanized
  CDS (1)..(357)
caggttcagctgcaagagtctggccctggcctggtcaagccttctcagaccctgtctctgacctgcagcgtgaccggctactccatcacctccgactactactggcactggatcagacagcctccaggcaaaggcctggaatggatcgcctacatcagatacgacggccggaacgacagcaaccccagcctgaagaacagagtgaccatcagccgggacacctccaagaaccagttctccctgaagctgtcctccgtgaccgctgctgataccgccgtgtactactgcgccagagaggactacgcctcctcctcctttgattactggggccagggcaccctggtcaccgttagttct

SEQ ID NO: 18 - protein, 119 aa, Artificial Sequence
  Synthetic Construct
QVQLQESGPGLVKPSQTLSLTCSVTGYSITSDYYWHWIRQPPGKGLEWIAYIRYDGRNDSNPSLKNRVTISRDTSKNQFSLKLSSVTAADTAVYYCAREDYASSSFDYWGQGTLVTVSS

SEQ ID NO: 19 - DNA, 324 bp, Artificial Sequence
  mouse antibody/ humanized
  CDS (1)..(324)
gacatccagatgacccagtctccatcctctctgtccgcctctgtgggcgacagagtgaccatcacctgtcggccttccgagaacatctactccaacctggcctggtatcagcagaagcctggcaaggctcctaagctgctggtgtacgccgctaccaatctggctgatggcgtgccctctagattctccggctctggctctggcaccgactataccctgacaatctccagcctgcagcctgaggatatcgccacctactactgccagcacttctgggacagccctccaacctttggccagggcaccaagctggaaatcaagcgt

SEQ ID NO: 20 - protein, 108 aa, Artificial Sequence
  Synthetic Construct
DIQMTQSPSSLSASVGDRVTITCRPSENIYSNLAWYQQKPGKAPKLLVYAATNLADGVPSRFSGSGSGTDYTLTISSLQPEDIATYYCQHFWDSPPTFGQGTKLEIKR

SEQ ID NO: 21 - DNA, 1350 bp, Artificial Sequence
  modified antibody
  CDS (1)..(1350)
caggtccagctgcaagagtctggccctggactggtcaagccttctggcaccctgtctctgacatgtgctgtgtccggcggctccatctcctcctctaattggtggtcttgggtccgacagcctcctggcaaaggactggaatggatcggcgagatctaccactccggcaacaccaactacaaccccagcctgaagtccagagtgaccgtgtccgtggacaagtccaagaaccagttctccctgaagctgacctctgtgaccgctgccgataccgccgtgtactactgtgctagagatgtgtctggcggagtgaattggttcgatccttggggccagggcacactggttaccgtgtcctctgcttctaccaagggaccctctgtgttccctctggctccttccagcaagtctacctctggtggaaccgctgctctgggctgcctggtcaaggattactttcctgagcctgtgacagtgtcctggaactctggtgctctgacatccggcgtgcacacctttccagctgtgctgcagtcctctggcctgtactctctgtcctctgtcgtgaccgtgccttctagctctctgggcacccagacctacatctgcaacgtgaaccacaagccttccaacaccaaggtggacaagaaggtggaacccaagtcctgcgacaagacccacacctgtcctccatgtcctgctccagaagctgctggcggtccctccgttttcctgtttccacctaagcctaaggacaccctgatgatctctcggacccctgaagtgacatgcgtggtggtggatgtgtcccacgaggatcccgaagtgaagttcaattggtacgtggacggcgtggaagtgcacaacgccaagaccaagcctagagaggaacagtacaactccacctacagagtggtgtccgtgctgaccgtgctgcaccaggattggctgaacggcaaagagtacaagtgcaaggtgtccaacaaggccctgcctgctcctatcgaaaagaccatctccaaggctaagggccagcctcgggaacctcaggtttacacactgcctccatctcgggacgagctgaccaagaatcaggtgtccctgtcttgcgccgtgaagggcttctacccttctgatatcgccgtggaatgggagtccaacggccagcctgagaacaactacaagacaacccctcctgtgctggactccgacggctcattcttcctggtgtccaagctgacagtggataagtctcggtggcagcagggcaacgtgttctcctgttctgtgatgcacgaggccctgcacaaccactacacccagaagagtctgtctctgtcccctggcaag

SEQ ID NO: 22 - protein, 450 aa, Artificial Sequence
  Synthetic Construct
QVQLQESGPGLVKPSGTLSLTCAVSGGSISSSNWWSWVRQPPGKGLEWIGEIYHSGNTNYNPSLKSRVTVSVDKSKNQFSLKLTSVTAADTAVYYCARDVSGGVNWFDPWGQGTLVTVSSASTKGPSVFPLAPSSKSTSGGTAALGCLVKDYFPEPVTVSWNSGALTSGVHTFPAVLQSSGLYSLSSVVTVPSSSLGTQTYICNVNHKPSNTKVDKKVEPKSCDKTHTCPPCPAPEAAGGPSVFLFPPKPKDTLMISRTPEVTCVVVDVSHEDPEVKFNWYVDGVEVHNAKTKPREEQYNSTYRVVSVLTVLHQDWLNGKEYKCKVSNKALPAPIEKTISKAKGQPREPQVYTLPPSRDELTKNQVSLSCAVKGFYPSDIAVEWESNGQPENNYKTTPPVLDSDGSFFLVSKLTVDKSRWQQGNVFSCSVMHEALHNHYTQKSLSLSPGK

SEQ ID NO: 23 - DNA, 648 bp, Artificial Sequence
  modified antibody
  CDS (1)..(648)
aactttatgctgacccagcctcactccgtgtccgagtctccaggcaagaccgtgaccatctcctgtaccagatcctccggctctatcgcctccaactacgtgcagtggtatcagcagaggcctggctctgctcctaccaccgtgatctacgaggacaaccagaggccttctggcgtgcccgataggttctctggctccatcgactcctcttccaactccgcctctctgaccatcagcggcctgaaaaccgaggacgaggccgactactactgccagtcctacgactcttccaccgtggtgtttggcggcggaacaaagctgacagtgctgggccagcctaaggccaatcctaccgtgacactgttccctccatcctccgaggaactgcaggctaacaaggctaccctcgtgtgcctgatctccgatttttaccctggcgctgtgaccgtggcttggaaggctgatggatctcctgtgaaggccggcgtggaaaccaccaagcctagcaagcagtccaacaacaaatacgccgcctcctcctacctgtctctgacccctgaacagtggaagtcccaccggtcctactcttgccaagtgacccatgagggcagcaccgtggaaaagacagtggcccctaccgagtgctct

SEQ ID NO: 24 - protein, 216 aa, Artificial Sequence
  Synthetic Construct
NFMLTQPHSVSESPGKTVTISCTRSSGSIASNYVQWYQQRPGSAPTTVIYEDNQRPSGVPDRFSGSIDSSSNSASLTISGLKTEDEADYYCQSYDSSTVVFGGGTKLTVLGQPKANPTVTLFPPSSEELQANKATLVCLISDFYPGAVTVAWKADGSPVKAGVETTKPSKQSNNKYAASSYLSLTPEQWKSHRSYSCQVTHEGSTVEKTVAPTECS

SEQ ID NO: 25 - DNA, 1353 bp, Artificial Sequence
  mouse antibody/ humanized
  CDS (1)..(1353)
gaagttcagctggttcagtctggcgccgaagtgaagaagcctggcgagtccctgaagatctcctgcaaaggctccggctacacctacaccagctactggatgaactgggtccgacagatgcctggcaaaggcctggaatggatgggcagaatcgacccctacgactccgagacacactacgaccagaaattcaaggaccaagtgaccctgagcgtggacaagtccatctccaccgcttacctgcagtggtcctctctgaaggcctctgacaccgccatgtactactgtgctggcggcatcaccaccatcctcggcggctactttgattactggggccagggcacactggtcaccgtttcttccgctagcaccaagggacccagcgtgttccctctggctccttccagcaagtctacctctggcggaacagctgctctgggctgcctggtcaaggactactttcctgagcctgtgaccgtgtcctggaactctggcgctctgacatctggcgtgcacacctttccagctgtgctgcagtcctccggcctgtactctctgtcctctgtcgtgaccgtgccttccagctctctgggaacccagacctacatctgcaatgtgaaccacaagccttccaacaccaaggtggacaagaaggtggaacccaagtcctgcgacaagacccacacctgtcctccatgtcctgctccagaagctgctggcggaccttccgtgtttctgttccctccaaagcctaaggacaccctgatgatctctcggacccctgaagtgacctgcgtggtggtggatgtgtctcacgaggacccagaagtgaagttcaattggtacgtggacggcgtggaagtgcacaacgccaagaccaagcctagagaggaacagtacaactccacctacagagtggtgtccgtgctgaccgtgctgcaccaggattggctgaacggcaaagagtacaagtgcaaggtgtccaacaaggccctgcctgctcctatcgaaaagaccatctccaaggccaagggccagcctagggaaccccaggtttacaccttgcctccatctcgggacgagctgaccaagaaccaggtgtccctgtcttgtgccgtgaagggcttctacccctccgatatcgctgtggaatgggagagcaatggccagcctgagaacaactacaagacaacccctcctgtgctggactccgacggctcattcttcctggtgtccaagctgacagtggataagtccagatggcagcagggcaacgtgttctcctgcagcgtgatgcacgaggccctgcacaatcactacacacagaagtctctgtctctgagccccggcaag

SEQ ID NO: 26 - protein, 451 aa, Artificial Sequence
  Synthetic Construct
EVQLVQSGAEVKKPGESLKISCKGSGYTYTSYWMNWVRQMPGKGLEWMGRIDPYDSETHYDQKFKDQVTLSVDKSISTAYLQWSSLKASDTAMYYCAGGITTILGGYFDYWGQGTLVTVSSASTKGPSVFPLAPSSKSTSGGTAALGCLVKDYFPEPVTVSWNSGALTSGVHTFPAVLQSSGLYSLSSVVTVPSSSLGTQTYICNVNHKPSNTKVDKKVEPKSCDKTHTCPPCPAPEAAGGPSVFLFPPKPKDTLMISRTPEVTCVVVDVSHEDPEVKFNWYVDGVEVHNAKTKPREEQYNSTYRVVSVLTVLHQDWLNGKEYKCKVSNKALPAPIEKTISKAKGQPREPQVYTLPPSRDELTKNQVSLSCAVKGFYPSDIAVEWESNGQPENNYKTTPPVLDSDGSFFLVSKLTVDKSRWQQGNVFSCSVMHEALHNHYTQKSLSLSPGK

SEQ ID NO: 27 - DNA, 645 bp, Artificial Sequence
  mouse antibody/ humanized
  CDS (1)..(645)
gacatccagatgacccagtctccatcctctctgtccgcctctgtgggcgacagagtgaccatcacctgtagagccagccaggacatctccaactacctgaactggtatcagcagaagcccggcaaggcccctaagctgctgatctactacacctctcggctgcactctggcgtgccctctagattttctggctccggctctggcaccgactataccctgacaatctccagcctgcagcctgaggacttcgccacctactattgccagcagggcaacaccctgcctccatacacatttggccagggcaccaaggtggaaatcaagcgtacggtggccgctccttccgtgttcatcttcccaccttccgacgagcagctgaagtccggcacagcttctgtcgtgtgcctgctgaacaacttctaccctcgggaagccaaggtgcagtggaaggtggacaatgccctgcagtccggcaactcccaagagtctgtgaccgagcaggactccaaggacagcacctacagcctgtcctccacactgaccctgtccaaggccgactacgagaagcacaaggtgtacgcctgcgaagtgacccatcagggcctgtctagccctgtgaccaagtctttcaaccggggcgagtgc

SEQ ID NO: 28 - protein, 215 aa, Artificial Sequence
  Synthetic Construct
DIQMTQSPSSLSASVGDRVTITCRASQDISNYLNWYQQKPGKAPKLLIYYTSRLHSGVPSRFSGSGSGTDYTLTISSLQPEDFATYYCQQGNTLPPYTFGQGTKVEIKRTVAAPSVFIFPPSDEQLKSGTASVVCLLNNFYPREAKVQWKVDNALQSGNSQESVTEQDSKDSTYSLSSTLTLSKADYEKHKVYACEVTHQGLSSPVTKSFNRGEC

SEQ ID NO: 29 - DNA, 1356 bp, Artificial Sequence
  mouse antibody/ humanized
  CDS (1)..(1356)
gaagtgcagctggttgaatctggcggcggattggttcagcctggcggatctctgagactgtcctgcaaggcttctggctacgcctacacctcctactggatgaactgggtccgacaggctcctggcaaaggactcgtgtgggtcggaagaatcgacccctacgactccgagacacactacaaccagaagttcaaggaccggttcaccctgagcgtggacaaggccaagtctaccacctacctgcagatgaactccctgagagccgaggacaccgccgtgtactattgcgctaccctgatcaccacactgagaggcgagggcgccatggaatattggggacagggaaccctggtcaccgtgtcctctgctagcaccaagggaccctctgtgttccctctggctccttccagcaagtccacctctggtggaacagctgctctgggctgcctggtcaaggactactttcctgagcctgtgaccgtgtcttggaactctggcgctctgacatctggcgtgcacacctttccagctgtgctgcagtcctccggcctgtactctctgtcctctgtcgtgaccgtgccttccagctctctgggaacccagacctacatctgcaatgtgaaccacaagccttccaacaccaaggtcgacaagaaggtggaacccaagtcctgcgacaagacccacacctgtcctccatgtcctgctccagaagctgctggcggcccttccgtgtttctgttccctccaaagcctaaggacaccctgatgatctctcggacccctgaagtgacctgcgtggtggtggatgtgtctcacgaggatcccgaagtgaagttcaattggtacgtggacggcgtggaagtgcacaacgccaagaccaagcctagagaggaacagtacaactccacctacagagtggtgtccgtgctgaccgtgctgcaccaggattggctgaacggcaaagagtacaagtgcaaggtgtccaacaaggccctgcctgctcctatcgaaaagaccatctctaaggccaagggccagcctcgggaacctcaggtttacaccttgcctccatctcgggacgagctgaccaagaaccaggtgtccctgtcttgtgccgtgaagggcttctacccctccgatatcgctgtggaatgggagagcaatggccagcctgagaacaactacaagacaacccctcctgtgctggactccgacggctcattcttcctggtgtccaagctgacagtggacaagtccagatggcagcagggcaacgtgttctcctgcagcgtgatgcacgaggccctgcacaatcactatacccagaagtctctgtctctgagccccggcaag

SEQ ID NO: 30 - protein, 452 aa, Artificial Sequence
  Synthetic Construct
EVQLVESGGGLVQPGGSLRLSCKASGYAYTSYWMNWVRQAPGKGLVWVGRIDPYDSETHYNQKFKDRFTLSVDKAKSTTYLQMNSLRAEDTAVYYCATLITTLRGEGAMEYWGQGTLVTVSSASTKGPSVFPLAPSSKSTSGGTAALGCLVKDYFPEPVTVSWNSGALTSGVHTFPAVLQSSGLYSLSSVVTVPSSSLGTQTYICNVNHKPSNTKVDKKVEPKSCDKTHTCPPCPAPEAAGGPSVFLFPPKPKDTLMISRTPEVTCVVVDVSHEDPEVKFNWYVDGVEVHNAKTKPREEQYNSTYRVVSVLTVLHQDWLNGKEYKCKVSNKALPAPIEKTISKAKGQPREPQVYTLPPSRDELTKNQVSLSCAVKGFYPSDIAVEWESNGQPENNYKTTPPVLDSDGSFFLVSKLTVDKSRWQQGNVFSCSVMHEALHNHYTQKSLSLSPGK

SEQ ID NO: 31 - DNA, 642 bp, Artificial Sequence
  mouse antibody/ humanized
  CDS (1)..(642)
gacctgcagatgacccagtctccttccagcctgtctgcctctgtgggcgacagagtgaccatcacatgcaaggccagccaggacgtgaacaccgccgttgcttggtatcagcagaagcctggcaaggcccctaagctgctgatctactgggcctccaccagacataccggcgtgccctctagattctccggctctggctctggcaccgactataccctgacaatctccagcctgcagcctgaggacttcgccacctactactgccagcagcactacagcacccctttcacctttggccagggcaccaaggtggaaatcaagcgtacggtggccgctccttccgtgttcatcttcccaccttccgacgagcagctgaagtccggcacagcttctgtcgtgtgcctgctgaacaacttctaccctcgggaagccaaggtgcagtggaaggtggacaatgccctgcagtccggcaactcccaagagtctgtgaccgagcaggactccaaggacagcacctatagcctgtcctccacactgaccctgtccaaggccgactacgagaagcacaaggtgtacgcctgcgaagtgacccatcagggcctgtctagtcccgtgaccaagtctttcaaccggggcgagtgc

SEQ ID NO: 32 - protein, 214 aa, Artificial Sequence
  Synthetic Construct
DLQMTQSPSSLSASVGDRVTITCKASQDVNTAVAWYQQKPGKAPKLLIYWASTRHTGVPSRFSGSGSGTDYTLTISSLQPEDFATYYCQQHYSTPFTFGQGTKVEIKRTVAAPSVFIFPPSDEQLKSGTASVVCLLNNFYPREAKVQWKVDNALQSGNSQESVTEQDSKDSTYSLSSTLTLSKADYEKHKVYACEVTHQGLSSPVTKSFNRGEC

SEQ ID NO: 33 - DNA, 1347 bp, Artificial Sequence
  mouse antibody/ humanized
  CDS (1)..(1347)
caggttcagctgcaagagtctggccctggcctggtcaagccttccgaaacactgtccctgacctgcagcgtgaccggctactctatcacctccgactactactggcactggatcagacagcctccaggcaaaggcctggaatggatcgcctacatcagatacgacggccggaacgactacaaccccagcctgaagaacagagtgaccatcagccgggacacctccaagaaccagttctccctgaagctgtcctccgtgaccgctgctgataccgccgtgtactactgcgccagagaggactacggctcctcctcctttgattactggggccagggcaccctggtcaccgttagttctgctagcaccaagggacccagcgtgttccctctggctccttccagcaagtctacctctggcggaacagctgctctgggctgtctggtcaaggactacttccctgagcctgtgaccgtgtcctggaactctggcgctctgacatctggcgtgcacacctttccagctgtgctgcagtcctccggcctgtactctctgtcctctgtcgtgaccgtgccttccagctctctgggaacccagacctacatctgcaatgtgaaccacaagcctagcaacaccaaggtggacaagaaggtggaacccaagtcctgcgacaagacccacacctgtcctccatgtcctgctccagaagctgctggcggcccttccgtgtttctgttccctccaaagcctaaggacaccctgatgatctctcggacccctgaagtgacctgcgtggtggtggatgtgtctcacgaggatcccgaagtgaagttcaattggtacgtggacggcgtggaagtgcacaacgccaagaccaagcctagagaggaacagtacaactccacctacagagtggtgtccgtgctgaccgtgctgcaccaggattggctgaacggcaaagagtacaagtgcaaggtgtccaacaaggccctgcctgctcctatcgaaaagaccatctccaaggctaagggccagcctcgggaacctcaggtgtacacattgcctccatctcgggacgagctgaccaagaatcaggtgtccctgtcttgcgccgtgaagggcttctacccttccgatatcgccgtggaatgggagtccaatggccagccagagaacaactacaagacaacccctcctgtgctggactccgacggctcattcttcctggtgtccaagctgacagtggacaagtccagatggcagcagggcaacgtgttctcctgctctgtgatgcacgaggccctgcacaaccactacacccagaagtctctgtctctgagccccggcaag

SEQ ID NO: 34 - protein, 449 aa, Artificial Sequence
  Synthetic Construct
QVQLQESGPGLVKPSETLSLTCSVTGYSITSDYYWHWIRQPPGKGLEWIAYIRYDGRNDYNPSLKNRVTISRDTSKNQFSLKLSSVTAADTAVYYCAREDYGSSSFDYWGQGTLVTVSSASTKGPSVFPLAPSSKSTSGGTAALGCLVKDYFPEPVTVSWNSGALTSGVHTFPAVLQSSGLYSLSSVVTVPSSSLGTQTYICNVNHKPSNTKVDKKVEPKSCDKTHTCPPCPAPEAAGGPSVFLFPPKPKDTLMISRTPEVTCVVVDVSHEDPEVKFNWYVDGVEVHNAKTKPREEQYNSTYRVVSVLTVLHQDWLNGKEYKCKVSNKALPAPIEKTISKAKGQPREPQVYTLPPSRDELTKNQVSLSCAVKGFYPSDIAVEWESNGQPENNYKTTPPVLDSDGSFFLVSKLTVDKSRWQQGNVFSCSVMHEALHNHYTQKSLSLSPGK

SEQ ID NO: 35 - DNA, 642 bp, Artificial Sequence
  mouse antibody/ humanized
  CDS (1)..(642)
gacatccagatgacccagtctccatcctctctgtccgcctctgtgggcgacagagtgaccatcacctgtcgggcctccgagaacatctactccaacctggcctggtatcagcagaagcctggcaaggctcctaagctgctggtgtacgccgctaccaatctggctgatggcgtgccctctagattctccggctctggctctggcaccgactataccctgacaatctccagcctgcagcctgaggacttcgccacctactactgccagcacttctgggacagccctccaacctttggccagggcaccaaggtggaaatcaagcgtacggtggccgctccttccgtgttcatcttcccaccttccgacgagcagctgaagtccggcacagcttctgtcgtgtgcctgctgaacaacttctaccctcgggaagccaaggtgcagtggaaggtggacaatgccctgcagtccggcaactcccaagagtctgtgaccgagcaggactccaaggacagcacctacagcctgtcctccacactgaccctgtccaaggccgactacgagaagcacaaggtgtacgcttgcgaagtgacccaccagggcctgtctagccctgtgaccaagtccttcaaccggggcgagtgc

SEQ ID NO: 36 - protein, 214 aa, Artificial Sequence
  Synthetic Construct
DIQMTQSPSSLSASVGDRVTITCRASENIYSNLAWYQQKPGKAPKLLVYAATNLADGVPSRFSGSGSGTDYTLTISSLQPEDFATYYCQHFWDSPPTFGQGTKVEIKRTVAAPSVFIFPPSDEQLKSGTASVVCLLNNFYPREAKVQWKVDNALQSGNSQESVTEQDSKDSTYSLSSTLTLSKADYEKHKVYACEVTHQGLSSPVTKSFNRGEC

SEQ ID NO: 37 - DNA, 1347 bp, Artificial Sequence
  mouse antibody/ humanized
  CDS (1)..(1347)
caggttcagctgcaagagtctggccctggcctggtcaagccttctcagaccctgtctctgacctgcagcgtgaccggctactccatcacctccgactactactggcactggatcagacagcctccaggcaaaggcctggaatggatcgcctacatcagatacgacggccggaacgacagcaaccccagcctgaagaacagagtgaccatcagccgggacacctccaagaaccagttctccctgaagctgtcctccgtgaccgctgctgataccgccgtgtactactgcgccagagaggactacgcctcctcctcctttgattactggggccagggcaccctggtcaccgttagttctgctagcaccaagggacccagcgtgttccctctggctccttccagcaagtctacctctggcggaacagctgctctgggctgtctggtcaaggactacttccctgagcctgtgaccgtgtcctggaactctggcgctctgacatctggcgtgcacacctttccagctgtgctgcagtcctccggcctgtactctctgtcctctgtcgtgaccgtgccttccagctctctgggaacccagacctacatctgcaatgtgaaccacaagccttccaacaccaaggtggacaagaaggtggaacccaagtcctgcgacaagacccacacctgtcctccatgtcctgctccagaagctgctggcggcccttccgtgtttctgttccctccaaagcctaaggacaccctgatgatctctcggacccctgaagtgacctgcgtggtggtggatgtgtctcacgaggatcccgaagtgaagttcaattggtacgtggacggcgtggaagtgcacaacgccaagaccaagcctagagaggaacagtacaactccacctacagagtggtgtccgtgctgaccgtgctgcaccaggattggctgaacggcaaagagtacaagtgcaaggtgtccaacaaggccctgcctgctcctatcgaaaagaccatctccaaggctaagggccagcctcgggaacctcaggtgtacacattgcctccatctcgggacgagctgaccaagaatcaggtgtccctgtcctgtgccgtgaagggcttctacccttccgatatcgccgtggaatgggagtccaatggccagccagagaacaactacaagacaacccctcctgtgctggactccgacggctcattcttcctggtgtccaagctgacagtggacaagtccagatggcagcagggcaacgtgttctcctgctctgtgatgcacgaggccctgcacaaccactacacccagaagagtctgtctctgtcccctggcaag

SEQ ID NO: 38 - protein, 449 aa, Artificial Sequence
  Synthetic Construct
QVQLQESGPGLVKPSQTLSLTCSVTGYSITSDYYWHWIRQPPGKGLEWIAYIRYDGRNDSNPSLKNRVTISRDTSKNQFSLKLSSVTAADTAVYYCAREDYASSSFDYWGQGTLVTVSSASTKGPSVFPLAPSSKSTSGGTAALGCLVKDYFPEPVTVSWNSGALTSGVHTFPAVLQSSGLYSLSSVVTVPSSSLGTQTYICNVNHKPSNTKVDKKVEPKSCDKTHTCPPCPAPEAAGGPSVFLFPPKPKDTLMISRTPEVTCVVVDVSHEDPEVKFNWYVDGVEVHNAKTKPREEQYNSTYRVVSVLTVLHQDWLNGKEYKCKVSNKALPAPIEKTISKAKGQPREPQVYTLPPSRDELTKNQVSLSCAVKGFYPSDIAVEWESNGQPENNYKTTPPVLDSDGSFFLVSKLTVDKSRWQQGNVFSCSVMHEALHNHYTQKSLSLSPGK

SEQ ID NO: 39 - DNA, 642 bp, Artificial Sequence
  mouse antibody/ humanized
  CDS (1)..(642)
gacatccagatgacccagtctccatcctctctgtccgcctctgtgggcgacagagtgaccatcacctgtcggccttccgagaacatctactccaacctggcctggtatcagcagaagcctggcaaggctcctaagctgctggtgtacgccgctaccaatctggctgatggcgtgccctctagattctccggctctggctctggcaccgactataccctgacaatctccagcctgcagcctgaggatatcgccacctactactgccagcacttctgggacagccctccaacctttggccagggcaccaagctggaaatcaagcgtacggtggccgctccttccgtgttcatcttcccaccttccgacgagcagctgaagtccggcacagcttctgtcgtgtgcctgctgaacaacttctaccctcgggaagccaaggtgcagtggaaggtggacaatgccctgcagtccggcaactcccaagagtctgtgaccgagcaggactccaaggacagcacctacagcctgtcctccacactgaccctgtccaaggccgactacgagaagcacaaggtgtacgcttgcgaagtgacccaccagggcctgtctagccctgtgaccaagtccttcaaccggggcgagtgc

SEQ ID NO: 40 - protein, 214 aa, Artificial Sequence
  Synthetic Construct
DIQMTQSPSSLSASVGDRVTITCRPSENIYSNLAWYQQKPGKAPKLLVYAATNLADGVPSRFSGSGSGTDYTLTISSLQPEDIATYYCQHFWDSPPTFGQGTKLEIKRTVAAPSVFIFPPSDEQLKSGTASVVCLLNNFYPREAKVQWKVDNALQSGNSQESVTEQDSKDSTYSLSSTLTLSKADYEKHKVYACEVTHQGLSSPVTKSFNRGEC

SEQ ID NO: 41 - DNA, 666 bp, Artificial Sequence
  modified Fc fragment
  CDS (1)..(666)
tgccctccatgtcctgctccagaagccgctggcggaccctctgtgtttctgttccctccaaagcctaaggacaccctgatgatctctcggacccctgaagtgacctgcgtggtggtggatgtgtctcacgaggatcccgaagtgaagttcaattggtacgtggacggcgtggaagtgcacaacgccaagaccaagcctagagaggaacagtacaactccacctacagagtggtgtccgtgctgaccgtgctgcaccaggattggctgaacggcaaagagtacaagtgcaaggtgtccaacaaggccctgcctgctcctatcgaaaagaccatctccaaggctaagggccagcctcgggaacctcaggtttacacactgcctccatctcgggacgagctgaccaagaatcaggtgtccctgtggtgcctggtcaagggcttctacccttccgatatcgccgtggaatgggagtccaatggccagcctgagaacaactacaagaccacacctcctgtgctggactccgacggctcattcttcctgtactccaagctgacagtggacaagtctcggtggcagcagggcaacgtgttctcctgttctgtgatgcacgaggccctgcacaaccactacacccagaagtccctgtctctgtcccctggcaaa

SEQ ID NO: 42 - protein, 222 aa, Artificial Sequence
  Synthetic Construct
CPPCPAPEAAGGPSVFLFPPKPKDTLMISRTPEVTCVVVDVSHEDPEVKFNWYVDGVEVHNAKTKPREEQYNSTYRVVSVLTVLHQDWLNGKEYKCKVSNKALPAPIEKTISKAKGQPREPQVYTLPPSRDELTKNQVSLWCLVKGFYPSDIAVEWESNGQPENNYKTTPPVLDSDGSFFLYSKLTVDKSRWQQGNVFSCSVMHEALHNHYTQKSLSLSPGK

SEQ ID NO: 43 - DNA, 1176 bp, Artificial Sequence
  codon optimized
  CDS (1)..(1176)
atgtcaacgatgaggctcctgacccttgctctgctgttcagctgctcagttgccagggctgcttgtgaccccaaaatcgtgaacattggcgccgtgctgtctaccagaaagcacgagcagatgtttagggaagccgtgaaccaggcaaacaagaggcatgggtcttggaaaattcagctgaatgcaacctctgtgacacacaagccaaatgccattcaaatggcactgtccgtctgcgaggacttgattagcagccaggtttacgccatactcgtgagccatcctcccacgcccaatgaccacttcactccaactcctgtttcctataccgctggcttttaccggattcctgtcttgggcctcaccacaagaatgagtatctacagtgacaagagcatacacctgagtttcctccgcactgtgcctccctatagtcaccagtcctctgtgtggttcgaaatgatgagggtctactcctggaatcacatcattctgttggtgtccgatgaccacgaaggacgtgcagcccagaaaaggctggaaactctgctcgaagaacgagagtcaaaagcggaaaaggtgctgcaattcgacccaggaacaaagaacgtcactgcgttgctgatggaggcaaaagagctggaagcacgggtgatcatcctcagcgcatcagaggacgatgccgccactgtgtatcgagctgctgcgatgctgaatatgacagggtccggctacgtctggcttgtcggcgagagagagattagcggtaatgctctgcggtatgctcccgatggcatcttggggcttcagctcatcaatggcaagaacgaaagcgcccatatttctgacgccgttggggtagtagcccaagcagttcacgagctgcttgagaaggagaacataaccgatccacctagagggtgtgtggggaacaccaacatttggaaaacaggaccgctgttcaaacgagttctgatgtctagcaagtatgctgatggcgtgacaggcagagtggagttcaacgaggatggtgatcggaaatttgctaactacagcattatgaatctgcaaaatcgcaaactggtacaggttgggatatacaatggaacccacgtgatcccgaacgaccggaagataatctggcctggaggcgaaacggagaaaccccgcggttat

SEQ ID NO: 44 - protein, 392 aa, Homo sapiens
MSTMRLLTLALLFSCSVARAACDPKIVNIGAVLSTRKHEQMFREAVNQANKRHGSWKIQLNATSVTHKPNAIQMALSVCEDLISSQVYAILVSHPPTPNDHFTPTPVSYTAGFYRIPVLGLTTRMSIYSDKSIHLSFLRTVPPYSHQSSVWFEMMRVYSWNHIILLVSDDHEGRAAQKRLETLLEERESKAEKVLQFDPGTKNVTALLMEAKELEARVIILSASEDDAATVYRAAAMLNMTGSGYVWLVGEREISGNALRYAPDGILGLQLINGKNESAHISDAVGVVAQAVHELLEKENITDPPRGCVGNTNIWKTGPLFKRVLMSSKYADGVTGRVEFNEDGDRKFANYSIMNLQNRKLVQVGIYNGTHVIPNDRKIIWPGGETEKPRGY

SEQ ID NO: 45 - DNA, 1350 bp, Artificial Sequence
  pathogenic anti-human NR1 antibody
  CDS (1)..(1350)
caggtccagctgcaagagtctggccctggactggtcaagccttctggcaccctgtctctgacatgtgctgtgtccggcggctccatctcctcctctaattggtggtcttgggtccgacagcctcctggcaaaggactggaatggatcggcgagatctaccactccggcaacaccaactacaaccccagcctgaagtccagagtgaccgtgtccgtggacaagtccaagaaccagttctccctgaagctgacctctgtgaccgctgccgataccgccgtgtactactgtgctagagatgtgtctggcggagtgaattggttcgatccttggggccagggcacactggttaccgtgtcctctgcttctaccaagggaccctctgtgttccctctggctccttccagcaagtctacctctggtggaaccgctgctctgggctgcctggtcaaggattactttcctgagcctgtgacagtgtcctggaactctggtgctctgacatccggcgtgcacacctttccagctgtgctgcagtcctctggcctgtactctctgtcctctgtcgtgaccgtgccttctagctctctgggcacccagacctacatctgcaacgtgaaccacaagccttccaacaccaaggtggacaagaaggtggaacccaagtcctgcgacaagacccacacctgtcctccatgtcctgctccagaactgctcggcggtccctccgttttcctgtttccacctaagcctaaggacaccctgatgatctctcggacccctgaagtgacatgcgtggtggtggatgtgtcccacgaggatcccgaagtgaagttcaattggtacgtggacggcgtggaagtgcacaacgccaagaccaagcctagagaggaacagtacaactccacctacagagtggtgtccgtgctgaccgtgctgcaccaggattggctgaacggcaaagagtacaagtgcaaggtgtccaacaaggccctgcctgctcctatcgaaaagaccatctccaaggctaagggccagcctcgggaacctcaggtttacacactgcctccatctcgggacgagctgaccaagaatcaggtgtccctgacctgcctcgtgaagggcttctacccttctgatatcgccgtggaatgggagtccaacggccagcctgagaacaactacaagacaacccctcctgtgctggactccgacggctcattcttcctgtactccaagctgacagtggataagtcccggtggcagcagggcaacgtgttctcttgttctgtgatgcacgaggccctgcacaaccactacacccagaagagtctgtctctgtcccctggcaag

SEQ ID NO: 46 - protein, 450 aa, Artificial Sequence
  Synthetic Construct
QVQLQESGPGLVKPSGTLSLTCAVSGGSISSSNWWSWVRQPPGKGLEWIGEIYHSGNTNYNPSLKSRVTVSVDKSKNQFSLKLTSVTAADTAVYYCARDVSGGVNWFDPWGQGTLVTVSSASTKGPSVFPLAPSSKSTSGGTAALGCLVKDYFPEPVTVSWNSGALTSGVHTFPAVLQSSGLYSLSSVVTVPSSSLGTQTYICNVNHKPSNTKVDKKVEPKSCDKTHTCPPCPAPELLGGPSVFLFPPKPKDTLMISRTPEVTCVVVDVSHEDPEVKFNWYVDGVEVHNAKTKPREEQYNSTYRVVSVLTVLHQDWLNGKEYKCKVSNKALPAPIEKTISKAKGQPREPQVYTLPPSRDELTKNQVSLTCLVKGFYPSDIAVEWESNGQPENNYKTTPPVLDSDGSFFLYSKLTVDKSRWQQGNVFSCSVMHEALHNHYTQKSLSLSPGK

SEQ ID NO: 47 - DNA, 648 bp, Artificial Sequence; identical to SEQ ID NO: 23
  Pathogenic anti-human NR1 antibody
  CDS (1)..(648)

SEQ ID NO: 48 - protein, 216 aa, Artificial Sequence; identical to SEQ ID NO: 24
  Synthetic Construct

SEQ ID NO: 49 - protein, 19 aa, Artificial Sequence
  Synthetic Construct
MEWSWVFLFFLSVTTGVHS

SEQ ID NO: 50 - protein, 20 aa, Artificial Sequence
  Synthetic Construct
MSVPTQVLGLLLLWLTDARC